European Patent Application EP 4 782 466 A1, published July 29, 2026. Title: 灭活冠状病毒的融合蛋白及其应用. Applicant: 山西锦波生物医药股份有限公司. Application CN. The sequence listing filed with the application follows.

SEQUENCE LISTING (13 sequences)

SEQ ID NO: 1 - protein, 615 aa, synthetic construct
MSSSSWLLLSLVAVTAAQSTIEEQAKTFLDKFNHEAEDLFYQSSLASWNYNTNITEENVQNMNNAGDKWSAFLKEQSTLAQMYPLQEIQNLTVKLQLQALQQNGSSVLSEDKSKRLNTILNTMSTIYSTGKVCNPDNPQECLLLEPGLNEIMANSLDYNERLWAWESWRSEVGKQLRPLYEEYVVLKNEMARANHYEDYGDYWRGDYEVNGVDGYDYSRGQLIEDVEHTFEEIKPLYEHLHAYVRAKLMNAYPSYISPIGCLPAHLLGDMWGRFWTNLYSLTVPFGQKPNIDVTDAMVDQAWDAQRIFKEAEKFFVSVGLPNMTQGFWENSMLTDPGNVQKAVCHPTAWDLGKGDFRILMCTKVTMDDFLTAHHEMGHIQYDMAYAAQPFLLRNGANEGFHEAVGEIMSLSAATPKHLKSIGLLSPDFQEDNETEINFLLKQALTIVGTLPFTYMLEKWRWMVFKGEIPKDQWMKKWWEMKREIVGVVEPVPHDETYCDPASLFHVSNDYSFIRYYTRTLYQFQFQEALCQAAKHEGPLHKCDISNSTEAGQKLFNMLRLGKSEPWTLALENVVGAKNMNVRPLLNYFEPLFTWLKDQNKNSFVGWSTDWSPYAD

SEQ ID NO: 2 - protein, 36 aa, synthetic construct
SLDQINVTFLDLEYEMKKLEEAIKKLEESYIDLKEL

SEQ ID NO: 3 - DNA, 1845 bp, synthetic construct
  source 1..1845: mol_type = other DNA
atgtcaagctcttcctggctccttctcagccttgttgctgtaactgctgctcagtccaccattgaggaacaggccaagacatttttggacaagtttaaccacgaagccgaagacctgttctatcaaagttcacttgcttcttggaattataacaccaatattactgaagagaatgtccaaaacatgaataatgctggggacaaatggtctgcctttttaaaggaacagtccacacttgcccaaatgtatccactacaagaaattcagaatctcacagtcaagcttcagctgcaggctcttcagcaaaatgggtcttcagtgctctcagaagacaagagcaaacggttgaacacaattctaaatacaatgagcaccatctacagtactggaaaagtttgtaacccagataatccacaagaatgcttattacttgaaccaggtttgaatgaaataatggcaaacagtttagactacaatgagaggctctgggcttgggaaagctggagatctgaggtcggcaagcagctgaggccattatatgaagagtatgtggtcttgaaaaatgagatggcaagagcaaatcattatgaggactatggggattattggagaggagactatgaagtaaatggggtagatggctatgactacagccgcggccagttgattgaagatgtggaacatacctttgaagagattaaaccattatatgaacatcttcatgcctatgtgagggcaaagttgatgaatgcctatccttcctatatcagtccaattggatgcctccctgctcatttgcttggtgatatgtggggtagattttggacaaatctgtactctttgacagttccctttggacagaaaccaaacatagatgttactgatgcaatggtggaccaggcctgggatgcacagagaatattcaaggaggccgagaagttctttgtatctgttggtcttcctaatatgactcaaggattctgggaaaattccatgctaacggacccaggaaatgttcagaaagcagtctgccatcccacagcttgggacctggggaagggcgacttcaggatccttatgtgcacaaaggtgacaatggacgacttcctgacagctcatcatgagatggggcatatccagtatgatatggcatatgctgcacaaccttttctgctaagaaatggagctaatgaaggattccatgaagctgttggggaaatcatgtcactttctgcagccacacctaagcatttaaaatccattggtcttctgtcacccgattttcaagaagacaatgaaacagaaatcaacttcctgctgaagcaggccctgaccattgttgggactctgccatttacttacatgttagagaagtggaggtggatggtctttaaaggggaaattcccaaagaccagtggatgaaaaagtggtgggagatgaagcgagagatagttggggtggtggaacctgtgccccatgatgaaacatactgtgaccccgcatctctgttccatgtttctaatgattactcattcattcgatattacacaaggaccctttaccaattccagtttcaagaagcactttgtcaagcagctaaacatgaaggccctctgcacaaatgtgacatctcaaactctacagaagctggacagaaactgttcaatatgctgaggcttggaaaatcagaaccctggaccctagcattggaaaatgttgtaggagcaaagaacatgaatgtaaggccactgctcaactactttgagcccttatttacctggctgaaagaccagaacaagaattcttttgtgggatggagtaccgactggagtccatatgcagac

SEQ ID NO: 4 - DNA, 108 bp, synthetic construct
  source 1..108: mol_type = other DNA
agcctggaccagatcaacgtgaccttcctggacctggagtacgagatgaagaagctggaggaggccatcaagaagctggaggagagctacatcgacctgaaggagctg

SEQ ID NO: 5 - protein, 692 aa, synthetic construct
MSSSSWLLLSLVAVTAAQSTIEEQAKTFLDKFNHEAEDLFYQSSLASWNYNTNITEENVQNMNNAGDKWSAFLKEQSTLAQMYPLQEIQNLTVKLQLQALQQNGSSVLSEDKSKRLNTILNTMSTIYSTGKVCNPDNPQECLLLEPGLNEIMANSLDYNERLWAWESWRSEVGKQLRPLYEEYVVLKNEMARANHYEDYGDYWRGDYEVNGVDGYDYSRGQLIEDVEHTFEEIKPLYEHLHAYVRAKLMNAYPSYISPIGCLPAHLLGDMWGRFWTNLYSLTVPFGQKPNIDVTDAMVDQAWDAQRIFKEAEKFFVSVGLPNMTQGFWENSMLTDPGNVQKAVCHPTAWDLGKGDFRILMCTKVTMDDFLTAHHEMGHIQYDMAYAAQPFLLRNGANEGFHEAVGEIMSLSAATPKHLKSIGLLSPDFQEDNETEINFLLKQALTIVGTLPFTYMLEKWRWMVFKGEIPKDQWMKKWWEMKREIVGVVEPVPHDETYCDPASLFHVSNDYSFIRYYTRTLYQFQFQEALCQAAKHEGPLHKCDISNSTEAGQKLFNMLRLGKSEPWTLALENVVGAKNMNVRPLLNYFEPLFTWLKDQNKNSFVGWSTDWSPYADGGGGSGGGGSGGGGSGGGGSGGGGSSLDQINVTFLDLEYEMKKLEEAIKKLEESYIDLKELLEVLFQGPHHHHHHHH

SEQ ID NO: 6 - protein, 36 aa, synthetic construct
NPGDINVTFLDLEYEMKKLEEAIKKLEESYIDLKKL

SEQ ID NO: 7 - protein, 676 aa, synthetic construct
MSSSSWLLLSLVAVTAAQSTIEEQAKTFLDKFNHEAEDLFYQSSLASWNYNTNITEENVQNMNNAGDKWSAFLKEQSTLAQMYPLQEIQNLTVKLQLQALQQNGSSVLSEDKSKRLNTILNTMSTIYSTGKVCNPDNPQECLLLEPGLNEIMANSLDYNERLWAWESWRSEVGKQLRPLYEEYVVLKNEMARANHYEDYGDYWRGDYEVNGVDGYDYSRGQLIEDVEHTFEEIKPLYEHLHAYVRAKLMNAYPSYISPIGCLPAHLLGDMWGRFWTNLYSLTVPFGQKPNIDVTDAMVDQAWDAQRIFKEAEKFFVSVGLPNMTQGFWENSMLTDPGNVQKAVCHPTAWDLGKGDFRILMCTKVTMDDFLTAHHEMGHIQYDMAYAAQPFLLRNGANEGFHEAVGEIMSLSAATPKHLKSIGLLSPDFQEDNETEINFLLKQALTIVGTLPFTYMLEKWRWMVFKGEIPKDQWMKKWWEMKREIVGVVEPVPHDETYCDPASLFHVSNDYSFIRYYTRTLYQFQFQEALCQAAKHEGPLHKCDISNSTEAGQKLFNMLRLGKSEPWTLALENVVGAKNMNVRPLLNYFEPLFTWLKDQNKNSFVGWSTDWSPYADGGGGSGGGGSGGGGSGGGGSGGGGSSLDQINVTFLDLEYEMKKLEEAIKKLEESYIDLKEL

SEQ ID NO: 8 - DNA, 2034 bp, synthetic construct
  source 1..2034: mol_type = other DNA
atgtcaagctcttcctggctccttctcagccttgttgctgtaactgctgctcagtccaccattgaggaacaggccaagacatttttggacaagtttaaccacgaagccgaagacctgttctatcaaagttcacttgcttcttggaattataacaccaatattactgaagagaatgtccaaaacatgaataatgctggggacaaatggtctgcctttttaaaggaacagtccacacttgcccaaatgtatccactacaagaaattcagaatctcacagtcaagcttcagctgcaggctcttcagcaaaatgggtcttcagtgctctcagaagacaagagcaaacggttgaacacaattctaaatacaatgagcaccatctacagtactggaaaagtttgtaacccagataatccacaagaatgcttattacttgaaccaggtttgaatgaaataatggcaaacagtttagactacaatgagaggctctgggcttgggaaagctggagatctgaggtcggcaagcagctgaggccattatatgaagagtatgtggtcttgaaaaatgagatggcaagagcaaatcattatgaggactatggggattattggagaggagactatgaagtaaatggggtagatggctatgactacagccgcggccagttgattgaagatgtggaacatacctttgaagagattaaaccattatatgaacatcttcatgcctatgtgagggcaaagttgatgaatgcctatccttcctatatcagtccaattggatgcctccctgctcatttgcttggtgatatgtggggtagattttggacaaatctgtactctttgacagttccctttggacagaaaccaaacatagatgttactgatgcaatggtggaccaggcctgggatgcacagagaatattcaaggaggccgagaagttctttgtatctgttggtcttcctaatatgactcaaggattctgggaaaattccatgctaacggacccaggaaatgttcagaaagcagtctgccatcccacagcttgggacctggggaagggcgacttcaggatccttatgtgcacaaaggtgacaatggacgacttcctgacagctcatcatgagatggggcatatccagtatgatatggcatatgctgcacaaccttttctgctaagaaatggagctaatgaaggattccatgaagctgttggggaaatcatgtcactttctgcagccacacctaagcatttaaaatccattggtcttctgtcacccgattttcaagaagacaatgaaacagaaatcaacttcctgctgaagcaggccctgaccattgttgggactctgccatttacttacatgttagagaagtggaggtggatggtctttaaaggggaaattcccaaagaccagtggatgaaaaagtggtgggagatgaagcgagagatagttggggtggtggaacctgtgccccatgatgaaacatactgtgaccccgcatctctgttccatgtttctaatgattactcattcattcgatattacacaaggaccctttaccaattccagtttcaagaagcactttgtcaagcagctaaacatgaaggccctctgcacaaatgtgacatctcaaactctacagaagctggacagaaactgttcaatatgctgaggcttggaaaatcagaaccctggaccctagcattggaaaatgttgtaggagcaaagaacatgaatgtaaggccactgctcaactactttgagcccttatttacctggctgaaagaccagaacaagaattcttttgtgggatggagtaccgactggagtccatatgcagacggaggaggaggaagcggaggaggaggatctagcctggaccagatcaacgtgaccttcctggacctggagtacgagatgaagaagctggaggaggccatcaagaagctggaggagagctacatcgacctgaaggagctgctggaagttctgttccagggcccgcatcaccatcatcaccatcaccattga

SEQ ID NO: 9 - DNA, 2079 bp, synthetic construct
  source 1..2079: mol_type = other DNA
atgtcaagctcttcctggctccttctcagccttgttgctgtaactgctgctcagtccaccattgaggaacaggccaagacatttttggacaagtttaaccacgaagccgaagacctgttctatcaaagttcacttgcttcttggaattataacaccaatattactgaagagaatgtccaaaacatgaataatgctggggacaaatggtctgcctttttaaaggaacagtccacacttgcccaaatgtatccactacaagaaattcagaatctcacagtcaagcttcagctgcaggctcttcagcaaaatgggtcttcagtgctctcagaagacaagagcaaacggttgaacacaattctaaatacaatgagcaccatctacagtactggaaaagtttgtaacccagataatccacaagaatgcttattacttgaaccaggtttgaatgaaataatggcaaacagtttagactacaatgagaggctctgggcttgggaaagctggagatctgaggtcggcaagcagctgaggccattatatgaagagtatgtggtcttgaaaaatgagatggcaagagcaaatcattatgaggactatggggattattggagaggagactatgaagtaaatggggtagatggctatgactacagccgcggccagttgattgaagatgtggaacatacctttgaagagattaaaccattatatgaacatcttcatgcctatgtgagggcaaagttgatgaatgcctatccttcctatatcagtccaattggatgcctccctgctcatttgcttggtgatatgtggggtagattttggacaaatctgtactctttgacagttccctttggacagaaaccaaacatagatgttactgatgcaatggtggaccaggcctgggatgcacagagaatattcaaggaggccgagaagttctttgtatctgttggtcttcctaatatgactcaaggattctgggaaaattccatgctaacggacccaggaaatgttcagaaagcagtctgccatcccacagcttgggacctggggaagggcgacttcaggatccttatgtgcacaaaggtgacaatggacgacttcctgacagctcatcatgagatggggcatatccagtatgatatggcatatgctgcacaaccttttctgctaagaaatggagctaatgaaggattccatgaagctgttggggaaatcatgtcactttctgcagccacacctaagcatttaaaatccattggtcttctgtcacccgattttcaagaagacaatgaaacagaaatcaacttcctgctgaagcaggccctgaccattgttgggactctgccatttacttacatgttagagaagtggaggtggatggtctttaaaggggaaattcccaaagaccagtggatgaaaaagtggtgggagatgaagcgagagatagttggggtggtggaacctgtgccccatgatgaaacatactgtgaccccgcatctctgttccatgtttctaatgattactcattcattcgatattacacaaggaccctttaccaattccagtttcaagaagcactttgtcaagcagctaaacatgaaggccctctgcacaaatgtgacatctcaaactctacagaagctggacagaaactgttcaatatgctgaggcttggaaaatcagaaccctggaccctagcattggaaaatgttgtaggagcaaagaacatgaatgtaaggccactgctcaactactttgagcccttatttacctggctgaaagaccagaacaagaattcttttgtgggatggagtaccgactggagtccatatgcagacggaggaggaggaagcggaggaggaggatctggaggaggaggaagcggaggaggaggatctggaggaggaggaagcagcctggaccagatcaacgtgaccttcctggacctggagtacgagatgaagaagctggaggaggccatcaagaagctggaggagagctacatcgacctgaaggagctgctggaagttctgttccagggcccgcatcaccatcatcaccatcaccattga

SEQ ID NO: 10 - DNA, 2094 bp, synthetic construct
  source 1..2094: mol_type = other DNA
atgtcaagctcttcctggctccttctcagccttgttgctgtaactgctgctcagtccaccattgaggaacaggccaagacatttttggacaagtttaaccacgaagccgaagacctgttctatcaaagttcacttgcttcttggaattataacaccaatattactgaagagaatgtccaaaacatgaataatgctggggacaaatggtctgcctttttaaaggaacagtccacacttgcccaaatgtatccactacaagaaattcagaatctcacagtcaagcttcagctgcaggctcttcagcaaaatgggtcttcagtgctctcagaagacaagagcaaacggttgaacacaattctaaatacaatgagcaccatctacagtactggaaaagtttgtaacccagataatccacaagaatgcttattacttgaaccaggtttgaatgaaataatggcaaacagtttagactacaatgagaggctctgggcttgggaaagctggagatctgaggtcggcaagcagctgaggccattatatgaagagtatgtggtcttgaaaaatgagatggcaagagcaaatcattatgaggactatggggattattggagaggagactatgaagtaaatggggtagatggctatgactacagccgcggccagttgattgaagatgtggaacatacctttgaagagattaaaccattatatgaacatcttcatgcctatgtgagggcaaagttgatgaatgcctatccttcctatatcagtccaattggatgcctccctgctcatttgcttggtgatatgtggggtagattttggacaaatctgtactctttgacagttccctttggacagaaaccaaacatagatgttactgatgcaatggtggaccaggcctgggatgcacagagaatattcaaggaggccgagaagttctttgtatctgttggtcttcctaatatgactcaaggattctgggaaaattccatgctaacggacccaggaaatgttcagaaagcagtctgccatcccacagcttgggacctggggaagggcgacttcaggatccttatgtgcacaaaggtgacaatggacgacttcctgacagctcatcatgagatggggcatatccagtatgatatggcatatgctgcacaaccttttctgctaagaaatggagctaatgaaggattccatgaagctgttggggaaatcatgtcactttctgcagccacacctaagcatttaaaatccattggtcttctgtcacccgattttcaagaagacaatgaaacagaaatcaacttcctgctgaagcaggccctgaccattgttgggactctgccatttacttacatgttagagaagtggaggtggatggtctttaaaggggaaattcccaaagaccagtggatgaaaaagtggtgggagatgaagcgagagatagttggggtggtggaacctgtgccccatgatgaaacatactgtgaccccgcatctctgttccatgtttctaatgattactcattcattcgatattacacaaggaccctttaccaattccagtttcaagaagcactttgtcaagcagctaaacatgaaggccctctgcacaaatgtgacatctcaaactctacagaagctggacagaaactgttcaatatgctgaggcttggaaaatcagaaccctggaccctagcattggaaaatgttgtaggagcaaagaacatgaatgtaaggccactgctcaactactttgagcccttatttacctggctgaaagaccagaacaagaattcttttgtgggatggagtaccgactggagtccatatgcagacggaggaggaggaagcggaggaggaggaagcggaggaggaggatctggaggaggaggaagcggaggaggaggatctggaggaggaggaagcagcctggaccagatcaacgtgaccttcctggacctggagtacgagatgaagaagctggaggaggccatcaagaagctggaggagagctacatcgacctgaaggagctgctggaagttctgttccagggcccgcatcaccatcatcaccatcaccattga

SEQ ID NO: 11 - DNA, 2109 bp, synthetic construct
  source 1..2109: mol_type = other DNA
atgtcaagctcttcctggctccttctcagccttgttgctgtaactgctgctcagtccaccattgaggaacaggccaagacatttttggacaagtttaaccacgaagccgaagacctgttctatcaaagttcacttgcttcttggaattataacaccaatattactgaagagaatgtccaaaacatgaataatgctggggacaaatggtctgcctttttaaaggaacagtccacacttgcccaaatgtatccactacaagaaattcagaatctcacagtcaagcttcagctgcaggctcttcagcaaaatgggtcttcagtgctctcagaagacaagagcaaacggttgaacacaattctaaatacaatgagcaccatctacagtactggaaaagtttgtaacccagataatccacaagaatgcttattacttgaaccaggtttgaatgaaataatggcaaacagtttagactacaatgagaggctctgggcttgggaaagctggagatctgaggtcggcaagcagctgaggccattatatgaagagtatgtggtcttgaaaaatgagatggcaagagcaaatcattatgaggactatggggattattggagaggagactatgaagtaaatggggtagatggctatgactacagccgcggccagttgattgaagatgtggaacatacctttgaagagattaaaccattatatgaacatcttcatgcctatgtgagggcaaagttgatgaatgcctatccttcctatatcagtccaattggatgcctccctgctcatttgcttggtgatatgtggggtagattttggacaaatctgtactctttgacagttccctttggacagaaaccaaacatagatgttactgatgcaatggtggaccaggcctgggatgcacagagaatattcaaggaggccgagaagttctttgtatctgttggtcttcctaatatgactcaaggattctgggaaaattccatgctaacggacccaggaaatgttcagaaagcagtctgccatcccacagcttgggacctggggaagggcgacttcaggatccttatgtgcacaaaggtgacaatggacgacttcctgacagctcatcatgagatggggcatatccagtatgatatggcatatgctgcacaaccttttctgctaagaaatggagctaatgaaggattccatgaagctgttggggaaatcatgtcactttctgcagccacacctaagcatttaaaatccattggtcttctgtcacccgattttcaagaagacaatgaaacagaaatcaacttcctgctgaagcaggccctgaccattgttgggactctgccatttacttacatgttagagaagtggaggtggatggtctttaaaggggaaattcccaaagaccagtggatgaaaaagtggtgggagatgaagcgagagatagttggggtggtggaacctgtgccccatgatgaaacatactgtgaccccgcatctctgttccatgtttctaatgattactcattcattcgatattacacaaggaccctttaccaattccagtttcaagaagcactttgtcaagcagctaaacatgaaggccctctgcacaaatgtgacatctcaaactctacagaagctggacagaaactgttcaatatgctgaggcttggaaaatcagaaccctggaccctagcattggaaaatgttgtaggagcaaagaacatgaatgtaaggccactgctcaactactttgagcccttatttacctggctgaaagaccagaacaagaattcttttgtgggatggagtaccgactggagtccatatgcagacggaggaggaggaagcggaggaggaggaagcggaggaggaggaagcggaggaggaggatctggaggaggaggaagcggaggaggaggatctggaggaggaggaagcagcctggaccagatcaacgtgaccttcctggacctggagtacgagatgaagaagctggaggaggccatcaagaagctggaggagagctacatcgacctgaaggagctgctggaagttctgttccagggcccgcatcaccatcatcaccatcaccattga

SEQ ID NO: 12 - protein, 46 aa, synthetic construct
SLDQINVTFLDLEYEMKKLEEAIKKLEESYIDLKELGSGGRRRRRR

SEQ ID NO: 13 - protein, 13 aa, synthetic construct
DCAWHLGELVWCT